European Patent Specification EP 3 490 573 B1, published February 7, 2024. Title: Devices, Systems and Methods for the Production of Humanized Gut Commensal Microbiota. Applicant: Subhadra, Bobban. Application TBA. The sequence listing filed with the application follows.

SEQUENCE LISTING (1 sequence)

SEQ ID NO: 1 - protein, 42 aa, homo sapiens
QGWLTFLKAAGQGTKDMWKAYSDMKEANYKKFRQILPCLGEL